European Patent Specification EP 3 238 727 B1, published January 18, 2023. Title: Non-aggregating immunostimulatory oligonucleotide. Applicant: NATIONAL INSTITUTES OF BIOMEDICAL INNOVATION, HEALTH AND NUTRITION GeneDesign, Inc. The sequence listing filed with the application follows.

SEQUENCE LISTING (85 sequences)

SEQ ID NO: 1 - DNA, 60 bp, artificial sequence
  D35(CG)G-dAs40
  phosphorothioate linkage (1)..(1)
  phosphorothioate linkage (18)..(59)
ggtgcatcgatgcaggggggaaaaaaaaaaaaaaaaaaaaaaaaaaaaaaaaaaaaaaaa

SEQ ID NO: 2 - DNA, 60 bp, artificial sequence
  D35(GC)G-dAs40
  phosphorothioate linkage (1)..(1)
  phosphorothioate linkage (18)..(59)
ggtgcatgcatgcaggggggaaaaaaaaaaaaaaaaaaaaaaaaaaaaaaaaaaaaaaaa

SEQ ID NO: 3 - DNA, 60 bp, artificial sequence
  D35(TG)G-dAs40
  phosphorothioate linkage (1)..(1)
  phosphorothioate linkage (18)..(59)
ggtgcattgatgcaggggggaaaaaaaaaaaaaaaaaaaaaaaaaaaaaaaaaaaaaaaa

SEQ ID NO: 4 - DNA, 60 bp, artificial sequence
  D35(CT)G-dAs40
  phosphorothioate linkage (1)..(1)
  phosphorothioate linkage (18)..(59)
ggtgcatctatgcaggggggaaaaaaaaaaaaaaaaaaaaaaaaaaaaaaaaaaaaaaaa

SEQ ID NO: 5 - DNA, 60 bp, artificial sequence
  D35(CG)A-dAs40
  phosphorothioate linkage (1)..(1)
  phosphorothioate linkage (18)..(59)
ggtgcatcgatgcaaaaaaaaaaaaaaaaaaaaaaaaaaaaaaaaaaaaaaaaaaaaaaa

SEQ ID NO: 6 - DNA, 60 bp, artificial sequence
  D35(GC)A-dAs40
  phosphorothioate linkage (1)..(1)
  phosphorothioate linkage (18)..(59)
ggtgcatgcatgcaaaaaaaaaaaaaaaaaaaaaaaaaaaaaaaaaaaaaaaaaaaaaaa

SEQ ID NO: 7 - DNA, 60 bp, artificial sequence
  D35(TG)A-dAs40
  phosphorothioate linkage (1)..(1)
  phosphorothioate linkage (18)..(59)
ggtgcattgatgcaaaaaaaaaaaaaaaaaaaaaaaaaaaaaaaaaaaaaaaaaaaaaaa

SEQ ID NO: 8 - DNA, 60 bp, artificial sequence
  D35(CT)A-dAs40
  phosphorothioate linkage (1)..(1)
  phosphorothioate linkage (18)..(59)
ggtgcatctatgcaaaaaaaaaaaaaaaaaaaaaaaaaaaaaaaaaaaaaaaaaaaaaaa

SEQ ID NO: 9 - DNA, 60 bp, artificial sequence
  D35(CG)T-dAs40
  phosphorothioate linkage (1)..(1)
  phosphorothioate linkage (18)..(59)
ggtgcatcgatgcattttttaaaaaaaaaaaaaaaaaaaaaaaaaaaaaaaaaaaaaaaa

SEQ ID NO: 10 - DNA, 60 bp, artificial sequence
  D35(GC)T-dAs40
  phosphorothioate linkage (1)..(1)
  phosphorothioate linkage (18)..(59)
ggtgcatgcatgcattttttaaaaaaaaaaaaaaaaaaaaaaaaaaaaaaaaaaaaaaaa

SEQ ID NO: 11 - DNA, 60 bp, artificial sequence
  D35(TG)T-dAs40
  phosphorothioate linkage (1)..(1)
  phosphorothioate linkage (18)..(59)
ggtgcattgatgcattttttaaaaaaaaaaaaaaaaaaaaaaaaaaaaaaaaaaaaaaaa

SEQ ID NO: 12 - DNA, 60 bp, artificial sequence
  D35(CT)T-dAs40
  phosphorothioate linkage (1)..(1)
  phosphorothioate linkage (18)..(59)
ggtgcatctatgcattttttaaaaaaaaaaaaaaaaaaaaaaaaaaaaaaaaaaaaaaaa

SEQ ID NO: 13 - DNA, 60 bp, artificial sequence
  D35(CG)C-dAs40
  phosphorothioate linkage (1)..(1)
  phosphorothioate linkage (18)..(59)
ggtgcatcgatgcaccccccaaaaaaaaaaaaaaaaaaaaaaaaaaaaaaaaaaaaaaaa

SEQ ID NO: 14 - DNA, 60 bp, artificial sequence
  D35(GC)C-dAs40
  phosphorothioate linkage (1)..(1)
  phosphorothioate linkage (18)..(59)
ggtgcatgcatgcaccccccaaaaaaaaaaaaaaaaaaaaaaaaaaaaaaaaaaaaaaaa

SEQ ID NO: 15 - DNA, 60 bp, artificial sequence
  D35(TG)C-dAs40
  phosphorothioate linkage (1)..(1)
  phosphorothioate linkage (18)..(59)
ggtgcattgatgcaccccccaaaaaaaaaaaaaaaaaaaaaaaaaaaaaaaaaaaaaaaa

SEQ ID NO: 16 - DNA, 60 bp, artificial sequence
  D35(CT)C-dAs40
  phosphorothioate linkage (1)..(1)
  phosphorothioate linkage (18)..(59)
ggtgcatctatgcaccccccaaaaaaaaaaaaaaaaaaaaaaaaaaaaaaaaaaaaaaaa

SEQ ID NO: 17 - DNA, 60 bp, artificial sequence; identical to SEQ ID NO: 9
  D35T-dA40
  phosphorothioate linkage (1)..(1)
  phosphorothioate linkage (18)..(20)

SEQ ID NO: 18 - DNA, 60 bp, artificial sequence
  D35T-dTs40
  phosphorothioate linkage (1)..(1)
  phosphorothioate linkage (18)..(59)
ggtgcatcgatgcatttttttttttttttttttttttttttttttttttttttttttttt

SEQ ID NO: 19 - DNA, 60 bp, artificial sequence; identical to SEQ ID NO: 18
  D35T-dT40
  phosphorothioate linkage (1)..(1)
  phosphorothioate linkage (18)..(20)

SEQ ID NO: 20 - DNA, 60 bp, artificial sequence
  D35T-dCs40
  phosphorothioate linkage (1)..(1)
  phosphorothioate linkage (18)..(59)
ggtgcatcgatgcattttttcccccccccccccccccccccccccccccccccccccccc

SEQ ID NO: 21 - DNA, 60 bp, artificial sequence; identical to SEQ ID NO: 20
  D35T-dC40
  phosphorothioate linkage (1)..(1)
  phosphorothioate linkage (18)..(20)

SEQ ID NO: 22 - DNA, 12 bp, artificial sequence
  D35core
tgcatcgatgca

SEQ ID NO: 23 - DNA, 52 bp, artificial sequence
  D35core-dAs40
  phosphorothioate linkage (12)..(51)
tgcatcgatgcaaaaaaaaaaaaaaaaaaaaaaaaaaaaaaaaaaaaaaaaa

SEQ ID NO: 24 - DNA, 58 bp, artificial sequence
  D35coreT-dAs40
  phosphorothioate linkage (16)..(57)
tgcatcgatgcattttttaaaaaaaaaaaaaaaaaaaaaaaaaaaaaaaaaaaaaaaa

SEQ ID NO: 25 - DNA, 22 bp, artificial sequence
  D35core-dAs10
  phosphorothioate linkage (12)..(21)
tgcatcgatgcaaaaaaaaaaa

SEQ ID NO: 26 - DNA, 32 bp, artificial sequence
  D35core-dAs20
  phosphorothioate linkage (12)..(31)
tgcatcgatgcaaaaaaaaaaaaaaaaaaaaa

SEQ ID NO: 27 - DNA, 42 bp, artificial sequence
  D35core-dAs30
  phosphorothioate linkage (12)..(41)
tgcatcgatgcaaaaaaaaaaaaaaaaaaaaaaaaaaaaaaa

SEQ ID NO: 28 - DNA, 52 bp, artificial sequence; identical to SEQ ID NO: 23
  D35core-dAs40
  phosphorothioate linkage (12)..(51)

SEQ ID NO: 29 - DNA, 40 bp, artificial sequence
  dAs40 tail
  phosphorothioate linkage (1)..(39)
aaaaaaaaaaaaaaaaaaaaaaaaaaaaaaaaaaaaaaaa

SEQ ID NO: 30 - DNA, 20 bp, artificial sequence
  K3
atcgactctcgagcgttctc

SEQ ID NO: 31 - DNA, 20 bp, artificial sequence
  D35
  phosphorothioate linkage (1)..(1)
  phosphorothioate linkage (18)..(19)
ggtgcatcgatgcagggggg

SEQ ID NO: 32 - DNA, 20 bp, artificial sequence
  D35A
  phosphorothioate linkage (1)..(1)
  phosphorothioate linkage (18)..(19)
ggtgcatcgatgcaaaaaaa

SEQ ID NO: 33 - DNA, 20 bp, artificial sequence
  D35T
  phosphorothioate linkage (1)..(1)
  phosphorothioate linkage (18)..(19)
ggtgcatcgatgcatttttt

SEQ ID NO: 34 - DNA, 14 bp, artificial sequence
  D35C
  phosphorothioate linkage (1)..(1)
  phosphorothioate linkage (18)..(19)
ggtgcatcgatgca

SEQ ID NO: 35 - DNA, 13 bp, artificial sequence
  D35core-dAs1
  phosphorothioate linkage (12)..(12)
tgcatcgatgcaa

SEQ ID NO: 36 - DNA, 14 bp, artificial sequence
  D35core-dAs2
  phosphorothioate linkage (12)..(13)
tgcatcgatgcaaa

SEQ ID NO: 37 - DNA, 15 bp, artificial sequence
  D35core-dAs3
  phosphorothioate linkage (12)..(14)
tgcatcgatgcaaaa

SEQ ID NO: 38 - DNA, 16 bp, artificial sequence
  D35core-dAs4
  phosphorothioate linkage (12)..(15)
tgcatcgatgcaaaaa

SEQ ID NO: 39 - DNA, 17 bp, artificial sequence
  D35core-dAs5
  phosphorothioate linkage (12)..(16)
tgcatcgatgcaaaaaa

SEQ ID NO: 40 - DNA, 18 bp, artificial sequence
  D35core-dAs6
  phosphorothioate linkage (12)..(17)
tgcatcgatgcaaaaaaa

SEQ ID NO: 41 - DNA, 19 bp, artificial sequence
  D35core-dAs7
  phosphorothioate linkage (12)..(18)
tgcatcgatgcaaaaaaaa

SEQ ID NO: 42 - DNA, 20 bp, artificial sequence
  D35core-dAs8
  phosphorothioate linkage (12)..(19)
tgcatcgatgcaaaaaaaaa

SEQ ID NO: 43 - DNA, 21 bp, artificial sequence
  D35core-dAs9
  phosphorothioate linkage (12)..(20)
tgcatcgatgcaaaaaaaaaa

SEQ ID NO: 44 - DNA, 22 bp, artificial sequence
  D35core-dAs10
  phosphorothioate linkage (12)..(21)
tgcatcgatgcaaaaaaaaaaa

SEQ ID NO: 45 - DNA, 32 bp, artificial sequence; identical to SEQ ID NO: 26
  D35core-dAs20
  phosphorothioate linkage (12)..(31)

SEQ ID NO: 46 - DNA, 72 bp, artificial sequence
  D35core-dAs60
  phosphorothioate linkage (12)..(71)
tgcatcgatgcaaaaaaaaaaaaaaaaaaaaaaaaaaaaaaaaaaaaaaaaaaaaaaaaaaaaaaaaaaaaa

SEQ ID NO: 47 - DNA, 92 bp, artificial sequence
  D35core-dAs80
  phosphorothioate linkage (12)..(91)
tgcatcgatgcaaaaaaaaaaaaaaaaaaaaaaaaaaaaaaaaaaaaaaaaaaaaaaaaaaaaaaaaaaaaaaaaaaaaaaaaaaaaaaaaa

SEQ ID NO: 48 - DNA, 112 bp, artificial sequence
  D35core-dAs100
  phosphorothioate linkage (12)..(111)
tgcatcgatgcaaaaaaaaaaaaaaaaaaaaaaaaaaaaaaaaaaaaaaaaaaaaaaaaaaaaaaaaaaaaaaaaaaaaaaaaaaaaaaaaaaaaaaaaaaaaaaaaaaaaa

SEQ ID NO: 49 - DNA, 52 bp, artificial sequence; identical to SEQ ID NO: 23
  D35core-dAs40(S100%)
  phosphorothioate linkage (12)..(51)

SEQ ID NO: 50 - DNA, 52 bp, artificial sequence; identical to SEQ ID NO: 23
  D35core-dAs40(S50%)
  phosphorothioate linkage (12)..(12)
  phosphorothioate linkage (14)..(14)
  phosphorothioate linkage (16)..(16)
  phosphorothioate linkage (18)..(18)
  phosphorothioate linkage (20)..(20)
  phosphorothioate linkage (22)..(22)
  phosphorothioate linkage (24)..(24)
  phosphorothioate linkage (26)..(26)
  phosphorothioate linkage (28)..(28)
  phosphorothioate linkage (30)..(30)
  phosphorothioate linkage (32)..(32)
  phosphorothioate linkage (34)..(34)
  phosphorothioate linkage (36)..(36)
  phosphorothioate linkage (38)..(38)
  phosphorothioate linkage (40)..(40)
  phosphorothioate linkage (42)..(42)
  phosphorothioate linkage (44)..(44)
  phosphorothioate linkage (46)..(46)
  phosphorothioate linkage (48)..(48)
  phosphorothioate linkage (50)..(50)

SEQ ID NO: 51 - DNA, 52 bp, artificial sequence; identical to SEQ ID NO: 23
  D35core-dAs40(S35%)
  phosphorothioate linkage (12)..(12)
  phosphorothioate linkage (15)..(15)
  phosphorothioate linkage (18)..(18)
  phosphorothioate linkage (21)..(21)
  phosphorothioate linkage (24)..(24)
  phosphorothioate linkage (27)..(27)
  phosphorothioate linkage (30)..(30)
  phosphorothioate linkage (33)..(33)
  phosphorothioate linkage (36)..(36)
  phosphorothioate linkage (39)..(39)
  phosphorothioate linkage (42)..(42)
  phosphorothioate linkage (45)..(45)
  phosphorothioate linkage (48)..(48)

SEQ ID NO: 52 - DNA, 52 bp, artificial sequence; identical to SEQ ID NO: 23
  D35core-dAs40(S25%)
  phosphorothioate linkage (12)..(12)
  phosphorothioate linkage (16)..(16)
  phosphorothioate linkage (20)..(20)
  phosphorothioate linkage (24)..(24)
  phosphorothioate linkage (28)..(28)
  phosphorothioate linkage (32)..(32)
  phosphorothioate linkage (36)..(36)
  phosphorothioate linkage (40)..(40)
  phosphorothioate linkage (44)..(44)
  phosphorothioate linkage (48)..(48)

SEQ ID NO: 53 - DNA, 52 bp, artificial sequence; identical to SEQ ID NO: 23
  D35core-dAs40(S20%)
  phosphorothioate linkage (12)..(12)
  phosphorothioate linkage (17)..(17)
  phosphorothioate linkage (22)..(22)
  phosphorothioate linkage (27)..(27)
  phosphorothioate linkage (32)..(32)
  phosphorothioate linkage (37)..(37)
  phosphorothioate linkage (42)..(42)
  phosphorothioate linkage (47)..(47)

SEQ ID NO: 54 - DNA, 52 bp, artificial sequence; identical to SEQ ID NO: 23
  D35core-dAs40(S15%)
  phosphorothioate linkage (12)..(12)
  phosphorothioate linkage (19)..(19)
  phosphorothioate linkage (26)..(26)
  phosphorothioate linkage (33)..(33)
  phosphorothioate linkage (40)..(40)
  phosphorothioate linkage (47)..(47)

SEQ ID NO: 55 - DNA, 20 bp, artificial sequence
  A2216
  phosphorothioate linkage (1)..(2)
  phosphorothioate linkage (14)..(19)
gggggacgatcgtcgggggg

SEQ ID NO: 56 - DNA, 10 bp, artificial sequence
  A2216core
gacgatcgtc

SEQ ID NO: 57 - DNA, 21 bp, artificial sequence
  A2336
  phosphorothioate linkage (1)..(3)
  phosphorothioate linkage (15)..(20)
ggggacgacgtcgtggggggg

SEQ ID NO: 58 - DNA, 10 bp, artificial sequence
  A2336core
acgacgtcgt

SEQ ID NO: 59 - DNA, 24 bp, artificial sequence
  B2006(PS)
  phosphorothioate linkage (1)..(23)
tcgtcgttttgtcgttttgtcgtt

SEQ ID NO: 60 - DNA, 24 bp, artificial sequence
  B2006(PO)
tcgtcgttttgtcgttttgtcgtt

SEQ ID NO: 61 - DNA, 22 bp, artificial sequence
  C2395(PS)
  phosphorothioate linkage (1)..(21)
tcgtcgttttcggcgcgcgccg

SEQ ID NO: 62 - DNA, 22 bp, artificial sequence
  C2395(PO)
tcgtcgttttcggcgcgcgccg

SEQ ID NO: 63 - DNA, 23 bp, artificial sequence
  P21889(PS)
  phosphorothioate linkage (1)..(22)
tcgtcgacgatcggcgcgcgccg

SEQ ID NO: 64 - DNA, 23 bp, artificial sequence
  P21889(PO)
tcgtcgacgatcggcgcgcgccg

SEQ ID NO: 65 - DNA, 20 bp, artificial sequence
  full length A2216
gggggacgatcgtcgggggg

SEQ ID NO: 66 - DNA, 21 bp, artificial sequence
  full length A2336
ggggacgacgtcgtggggggg

SEQ ID NO: 67 - DNA, 24 bp, artificial sequence
  CPG 7909
  phosphorothioate linkage (1)..(23)
tcgtcgttttgtcgttttgtcgtt

SEQ ID NO: 68 - DNA, 24 bp, artificial sequence
  PF-3512676
  phosphorothioate linkage (1)..(23)
tcgtcgttttgtcgttttgtcgtt

SEQ ID NO: 69 - DNA, 30 bp, artificial sequence
  CYT003-QBG10
gggggggggggacgatcgtcgggggggggg

SEQ ID NO: 70 - DNA, 22 bp, artificial sequence
  1018 ISS
  phosphorothioate linkage (1)..(21)
tgactgtgaacgttcgagatga

SEQ ID NO: 71 - DNA, 19 bp, artificial sequence
  Kappaproct (DIMS 0150)
  phosphorothioate linkage (1)..(3)
  phosphorothioate linkage (16)..(18)
ggaacagttcgtccatggc

SEQ ID NO: 72 - DNA, 60 bp, artificial sequence
  D35-dNs40
  phosphorothioate linkage (1)..(2)
  phosphorothioate linkage (18)..(59)
  misc_feature (21)..(60): n is a, c, g, t or u
ggtgcatcgatgcaggggggnnnnnnnnnnnnnnnnnnnnnnnnnnnnnnnnnnnnnnnn

SEQ ID NO: 73 - DNA, 20 bp, artificial sequence
  D35beta
  phosphorothioate linkage (1)..(2)
  phosphorothioate linkage (18)..(19)
ggtgcatcgatgcagggggg

SEQ ID NO: 74 - DNA, 60 bp, artificial sequence
  dAs40-D35
  phosphorothioate linkage (1)..(41)
  phosphorothioate linkage (58)..(59)
aaaaaaaaaaaaaaaaaaaaaaaaaaaaaaaaaaaaaaaaggtgcatcgatgcagggggg

SEQ ID NO: 75 - DNA, 80 bp, artificial sequence
  D35-dAs40-D35
  phosphorothioate linkage (1)..(1)
  phosphorothioate linkage (18)..(61)
  phosphorothioate linkage (78)..(79)
ggtgcatcgatgcaggggggaaaaaaaaaaaaaaaaaaaaaaaaaaaaaaaaaaaaaaaaggtgcatcgatgcagggggg

SEQ ID NO: 76 - DNA, 60 bp, artificial sequence
  A2216-dAs40
  phosphorothioate linkage (1)..(2)
  phosphorothioate linkage (14)..(19)
  phosphorothioate linkage (21)..(59)
gggggacgatcgtcggggggaaaaaaaaaaaaaaaaaaaaaaaaaaaaaaaaaaaaaaaa

SEQ ID NO: 77 - DNA, 50 bp, artificial sequence
  A2216core-dAs40
  phosphorothioate linkage (11)..(49)
gacgatcgtcaaaaaaaaaaaaaaaaaaaaaaaaaaaaaaaaaaaaaaaa

SEQ ID NO: 78 - DNA, 61 bp, artificial sequence
  A2336-dAs40
  phosphorothioate linkage (1)..(3)
  phosphorothioate linkage (15)..(20)
  phosphorothioate linkage (22)..(60)
ggggacgacgtcgtgggggggaaaaaaaaaaaaaaaaaaaaaaaaaaaaaaaaaaaaaaaa

SEQ ID NO: 79 - DNA, 50 bp, artificial sequence
  A2336core-dAs40
  phosphorothioate linkage (21)..(49)
acgacgtcgtaaaaaaaaaaaaaaaaaaaaaaaaaaaaaaaaaaaaaaaa

SEQ ID NO: 80 - DNA, 64 bp, artificial sequence
  B2006(PS)-dAs40
  phosphorothioate linkage (1)..(23)
  phosphorothioate linkage (25)..(63)
tcgtcgttttgtcgttttgtcgttaaaaaaaaaaaaaaaaaaaaaaaaaaaaaaaaaaaaaaaa

SEQ ID NO: 81 - DNA, 64 bp, artificial sequence; identical to SEQ ID NO: 80
  B2006(PO)-dAs40
  phosphorothioate linkage (25)..(63)

SEQ ID NO: 82 - DNA, 62 bp, artificial sequence
  C2395(PS)-dAs40
  phosphorothioate linkage (1)..(21)
  phosphorothioate linkage (23)..(61)
tcgtcgttttcggcgcgcgccgaaaaaaaaaaaaaaaaaaaaaaaaaaaaaaaaaaaaaaaa

SEQ ID NO: 83 - DNA, 62 bp, artificial sequence; identical to SEQ ID NO: 82
  C2395(PO)-dAs40
  phosphorothioate linkage (23)..(61)

SEQ ID NO: 84 - DNA, 63 bp, artificial sequence
  P21889(PS)-dAs40
  phosphorothioate linkage (1)..(22)
  phosphorothioate linkage (24)..(62)
tcgtcgacgatcggcgcgcgccgaaaaaaaaaaaaaaaaaaaaaaaaaaaaaaaaaaaaaaaa

SEQ ID NO: 85 - DNA, 63 bp, artificial sequence; identical to SEQ ID NO: 84
  P21889(PO)-dAs40
  phosphorothioate linkage (24)..(62)